European Patent Application EP 4 803 626 A1, published September 9, 2026. Title: 一种抑制补体MASP2基因表达的dsRNA分子及其应用. Applicant: 石药集团中奇制药技术(石家庄)有限公司. Application CN. The sequence listing filed with the application follows.

SEQUENCE LISTING (106 sequences)

SEQ ID NO: 1 - RNA, 21 nt, synthetic construct
  source 1..21: mol_type = other RNA
  modified_base 1: mod_base = gm
  modified_base 2: mod_base = cm
  modified_base 3: mod_base = um
  modified_base 4..5: mod_base = cm
  modified_base 6: mod_base = gm
  modified_base 7: mod_base = OTHER; note; note (original language) = 2'-fluoroadenosine
  modified_base 8: mod_base = cm
  modified_base 9: mod_base = OTHER; note = 2'-fluorouridine
  modified_base 10: mod_base = OTHER; note = 2'-fluoroadenosine
  modified_base 11: mod_base = OTHER; note = 2'-fluorouridine
  modified_base 12: mod_base = um
  modified_base 13..14: mod_base = cm
  modified_base 15..16: mod_base = OTHER; note = 2'-O-methyladenosine
  modified_base 17: mod_base = cm
  modified_base 18: mod_base = gm
  modified_base 19: mod_base = OTHER; note = 2'-O-methyladenosine
  modified_base 20: mod_base = gm
  modified_base 21: mod_base = OTHER; note = 2'-O-methyladenosine
  modified_base 1^2: mod_base = OTHER; note = phosphorothioate linkage
  modified_base 2^3: mod_base = OTHER; note = phosphorothioate linkage
  modified_base 19^20: mod_base = OTHER; note = phosphorothioate linkage
  modified_base 20^21: mod_base = OTHER; note = phosphorothioate linkage
gctccgactactccaacgaga

SEQ ID NO: 2 - RNA, 23 nt, synthetic construct
  source 1..23: mol_type = other RNA
  modified_base 1: mod_base = um
  modified_base 2: mod_base = OTHER; note = 2'-fluorocytidine
  modified_base 3: mod_base = um
  modified_base 4: mod_base = cm
  modified_base 5: mod_base = gm
  modified_base 6..7: mod_base = um
  modified_base 8..9: mod_base = gm
  modified_base 10: mod_base = OTHER; note = 2'-O-methyladenosine
  modified_base 11: mod_base = gm
  modified_base 12: mod_base = um
  modified_base 13: mod_base = OTHER; note = 2'-O-methyladenosine
  modified_base 14: mod_base = OTHER; note = 2'-fluoroguanosine
  modified_base 15: mod_base = um
  modified_base 16: mod_base = OTHER; note = 2'-fluorocytidine
  modified_base 17..18: mod_base = gm
  modified_base 19: mod_base = OTHER; note = 2'-O-methyladenosine
  modified_base 20: mod_base = gm
  modified_base 21: mod_base = cm
  modified_base 22..23: mod_base = gm
  modified_base 1^2: mod_base = OTHER; note = phosphorothioate linkage
  modified_base 2^3: mod_base = OTHER; note = phosphorothioate linkage
  modified_base 21^22: mod_base = OTHER; note = phosphorothioate linkage
  modified_base 22^23: mod_base = OTHER; note = phosphorothioate linkage
tctcgttggagtagtcggagcgg

SEQ ID NO: 3 - RNA, 21 nt, synthetic construct
  source 1..21: mol_type = other RNA
  modified_base 1: mod_base = um
  modified_base 2: mod_base = OTHER; note = 2'-O-methyladenosine
  modified_base 3: mod_base = um
  modified_base 4..5: mod_base = cm
  modified_base 6: mod_base = gm
  modified_base 7: mod_base = OTHER; note = 2'-fluoroadenosine
  modified_base 8: mod_base = um
  modified_base 9..10: mod_base = OTHER; note = 2'-fluoroguanosine
  modified_base 11: mod_base = OTHER; note = 2'-fluorocytidine
  modified_base 12: mod_base = gm
  modified_base 13..14: mod_base = cm
  modified_base 15: mod_base = OTHER; note = 2'-O-methyladenosine
  modified_base 16..17: mod_base = cm
  modified_base 18: mod_base = um
  modified_base 19..20: mod_base = OTHER; note = 2'-O-methyladenosine
  modified_base 21: mod_base = um
  modified_base 1^2: mod_base = OTHER; note = phosphorothioate linkage
  modified_base 2^3: mod_base = OTHER; note = phosphorothioate linkage
  modified_base 19^20: mod_base = OTHER; note = phosphorothioate linkage
  modified_base 20^21: mod_base = OTHER; note = phosphorothioate linkage
tatccgatggcgccacctaat

SEQ ID NO: 4 - RNA, 23 nt, synthetic construct
  source 1..23: mol_type = other RNA
  modified_base 1: mod_base = OTHER; note = 2'-O-methyladenosine
  modified_base 2: mod_base = OTHER; note = 2'-fluorouridine
  modified_base 3: mod_base = um
  modified_base 4: mod_base = OTHER; note = 2'-O-methyladenosine
  modified_base 5..6: mod_base = gm
  modified_base 7: mod_base = um
  modified_base 8..9: mod_base = gm
  modified_base 10: mod_base = cm
  modified_base 11: mod_base = gm
  modified_base 12..13: mod_base = cm
  modified_base 14: mod_base = OTHER; note = 2'-fluoroadenosine
  modified_base 15: mod_base = um
  modified_base 16: mod_base = OTHER; note = 2'-fluorocytidine
  modified_base 17..18: mod_base = gm
  modified_base 19: mod_base = OTHER; note = 2'-O-methyladenosine
  modified_base 20: mod_base = um
  modified_base 21..22: mod_base = OTHER; note = 2'-O-methyladenosine
  modified_base 23: mod_base = gm
  modified_base 1^2: mod_base = OTHER; note = phosphorothioate linkage
  modified_base 2^3: mod_base = OTHER; note = phosphorothioate linkage
  modified_base 21^22: mod_base = OTHER; note = phosphorothioate linkage
  modified_base 22^23: mod_base = OTHER; note = phosphorothioate linkage
attaggtggcgccatcggataag

SEQ ID NO: 5 - RNA, 21 nt, synthetic construct
  source 1..21: mol_type = other RNA
  modified_base 1: mod_base = cm
  modified_base 2: mod_base = OTHER; note = 2'-O-methyladenosine
  modified_base 3..4: mod_base = cm
  modified_base 5: mod_base = gm
  modified_base 6: mod_base = um
  modified_base 7: mod_base = OTHER; note = 2'-fluoroadenosine
  modified_base 8: mod_base = OTHER; note = 2'-O-methyladenosine
  modified_base 9: mod_base = OTHER; note = 2'-fluorocytidine
  modified_base 10..11: mod_base = OTHER; note = 2'-fluoroadenosine
  modified_base 12: mod_base = gm
  modified_base 13: mod_base = cm
  modified_base 14: mod_base = gm
  modified_base 15: mod_base = cm
  modified_base 16: mod_base = OTHER; note = 2'-O-methyladenosine
  modified_base 17..18: mod_base = cm
  modified_base 19: mod_base = um
  modified_base 20: mod_base = gm
  modified_base 21: mod_base = OTHER; note = 2'-O-methyladenosine
  modified_base 1^2: mod_base = OTHER; note = phosphorothioate linkage
  modified_base 2^3: mod_base = OTHER; note = phosphorothioate linkage
  modified_base 19^20: mod_base = OTHER; note = phosphorothioate linkage
  modified_base 20^21: mod_base = OTHER; note = phosphorothioate linkage
caccgtaacaagcgcacctga

SEQ ID NO: 6 - RNA, 23 nt, synthetic construct
  source 1..23: mol_type = other RNA
  modified_base 1: mod_base = um
  modified_base 2: mod_base = OTHER; note = 2'-fluorocytidine
  modified_base 3: mod_base = OTHER; note = 2'-O-methyladenosine
  modified_base 4..5: mod_base = gm
  modified_base 6: mod_base = um
  modified_base 7: mod_base = gm
  modified_base 8: mod_base = cm
  modified_base 9: mod_base = gm
  modified_base 10: mod_base = cm
  modified_base 11..12: mod_base = um
  modified_base 13: mod_base = gm
  modified_base 14: mod_base = OTHER; note = 2'-fluorouridine
  modified_base 15: mod_base = um
  modified_base 16: mod_base = OTHER; note = 2'-fluoroadenosine
  modified_base 17: mod_base = cm
  modified_base 18..19: mod_base = gm
  modified_base 20: mod_base = um
  modified_base 21: mod_base = gm
  modified_base 22: mod_base = cm
  modified_base 23: mod_base = OTHER; note = 2'-O-methyladenosine
  modified_base 1^2: mod_base = OTHER; note = phosphorothioate linkage
  modified_base 2^3: mod_base = OTHER; note = phosphorothioate linkage
  modified_base 21^22: mod_base = OTHER; note = phosphorothioate linkage
  modified_base 22^23: mod_base = OTHER; note = phosphorothioate linkage
tcaggtgcgcttgttacggtgca

SEQ ID NO: 7 - RNA, 21 nt, synthetic construct
  source 1..21: mol_type = other RNA
  modified_base 1: mod_base = cm
  modified_base 2: mod_base = um
  modified_base 3: mod_base = OTHER; note = 2'-O-methyladenosine
  modified_base 4..5: mod_base = cm
  modified_base 6: mod_base = gm
  modified_base 7: mod_base = OTHER; note = 2'-fluorocytidine
  modified_base 8: mod_base = cm
  modified_base 9: mod_base = OTHER; note = 2'-fluorouridine
  modified_base 10: mod_base = OTHER; note = 2'-fluoroguanosine
  modified_base 11: mod_base = OTHER; note = 2'-fluorocytidine
  modified_base 12: mod_base = gm
  modified_base 13..14: mod_base = cm
  modified_base 15: mod_base = um
  modified_base 16: mod_base = cm
  modified_base 17: mod_base = um
  modified_base 18: mod_base = OTHER; note = 2'-O-methyladenosine
  modified_base 19: mod_base = cm
  modified_base 20..21: mod_base = um
  modified_base 1^2: mod_base = OTHER; note = phosphorothioate linkage
  modified_base 2^3: mod_base = OTHER; note = phosphorothioate linkage
  modified_base 19^20: mod_base = OTHER; note = phosphorothioate linkage
  modified_base 20^21: mod_base = OTHER; note = phosphorothioate linkage
ctaccgcctgcgcctctactt

SEQ ID NO: 8 - RNA, 23 nt, synthetic construct
  source 1..23: mol_type = other RNA
  modified_base 1: mod_base = OTHER; note = 2'-O-methyladenosine
  modified_base 2: mod_base = OTHER; note = 2'-fluoroadenosine
  modified_base 3: mod_base = gm
  modified_base 4: mod_base = um
  modified_base 5: mod_base = OTHER; note = 2'-O-methyladenosine
  modified_base 6: mod_base = gm
  modified_base 7: mod_base = OTHER; note = 2'-O-methyladenosine
  modified_base 8..9: mod_base = gm
  modified_base 10: mod_base = cm
  modified_base 11: mod_base = gm
  modified_base 12: mod_base = cm
  modified_base 13: mod_base = OTHER; note = 2'-O-methyladenosine
  modified_base 14: mod_base = OTHER; note = 2'-fluoroguanosine
  modified_base 15: mod_base = gm
  modified_base 16: mod_base = OTHER; note = 2'-fluorocytidine
  modified_base 17..18: mod_base = gm
  modified_base 19: mod_base = um
  modified_base 20: mod_base = OTHER; note = 2'-O-methyladenosine
  modified_base 21: mod_base = gm
  modified_base 22..23: mod_base = cm
  modified_base 1^2: mod_base = OTHER; note = phosphorothioate linkage
  modified_base 2^3: mod_base = OTHER; note = phosphorothioate linkage
  modified_base 21^22: mod_base = OTHER; note = phosphorothioate linkage
  modified_base 22^23: mod_base = OTHER; note = phosphorothioate linkage
aagtagaggcgcaggcggtagcc

SEQ ID NO: 9 - RNA, 21 nt, synthetic construct
  source 1..21: mol_type = other RNA
  modified_base 1..2: mod_base = cm
  modified_base 3: mod_base = gm
  modified_base 4: mod_base = um
  modified_base 5..6: mod_base = OTHER; note = 2'-O-methyladenosine
  modified_base 7: mod_base = OTHER; note = 2'-fluorocytidine
  modified_base 8: mod_base = OTHER; note = 2'-O-methyladenosine
  modified_base 9: mod_base = OTHER; note = 2'-fluoroadenosine
  modified_base 10: mod_base = OTHER; note = 2'-fluoroguanosine
  modified_base 11: mod_base = OTHER; note = 2'-fluorocytidine
  modified_base 12: mod_base = gm
  modified_base 13: mod_base = cm
  modified_base 14: mod_base = OTHER; note = 2'-O-methyladenosine
  modified_base 15..16: mod_base = cm
  modified_base 17: mod_base = um
  modified_base 18: mod_base = gm
  modified_base 19: mod_base = cm
  modified_base 20: mod_base = um
  modified_base 21: mod_base = OTHER; note = 2'-O-methyladenosine
  modified_base 1^2: mod_base = OTHER; note = phosphorothioate linkage
  modified_base 2^3: mod_base = OTHER; note = phosphorothioate linkage
  modified_base 19^20: mod_base = OTHER; note = phosphorothioate linkage
  modified_base 20^21: mod_base = OTHER; note = phosphorothioate linkage
ccgtaacaagcgcacctgcta

SEQ ID NO: 10 - RNA, 23 nt, synthetic construct
  source 1..23: mol_type = other RNA
  modified_base 1: mod_base = um
  modified_base 2: mod_base = OTHER; note = 2'-fluoroadenosine
  modified_base 3: mod_base = gm
  modified_base 4: mod_base = cm
  modified_base 5: mod_base = OTHER; note = 2'-O-methyladenosine
  modified_base 6..7: mod_base = gm
  modified_base 8: mod_base = um
  modified_base 10: mod_base = cm
  modified_base 11: mod_base = gm
  modified_base 12: mod_base = cm
  modified_base 13: mod_base = um
  modified_base 14: mod_base = OTHER; note = 2'-fluorouridine
  modified_base 15: mod_base = gm
  modified_base 16: mod_base = OTHER; note = 2'-fluorouridine
  modified_base 17: mod_base = um
  modified_base 18: mod_base = OTHER; note = 2'-O-methyladenosine
  modified_base 19: mod_base = cm
  modified_base 20..21: mod_base = gm
  modified_base 22: mod_base = um
  modified_base 23: mod_base = gm
  modified_base 1^2: mod_base = OTHER; note = phosphorothioate linkage
  modified_base 2^3: mod_base = OTHER; note = phosphorothioate linkage
  modified_base 21^22: mod_base = OTHER; note = phosphorothioate linkage
  modified_base 22^23: mod_base = OTHER; note = phosphorothioate linkage
tagcaggtgcgcttgttacggtg

SEQ ID NO: 11 - RNA, 21 nt, synthetic construct
  source 1..21: mol_type = other RNA
  modified_base 1..2: mod_base = cm
  modified_base 3: mod_base = um
  modified_base 4: mod_base = cm
  modified_base 5: mod_base = um
  modified_base 6: mod_base = gm
  modified_base 7: mod_base = OTHER; note = 2'-fluorocytidine
  modified_base 8: mod_base = gm
  modified_base 9: mod_base = OTHER; note = 2'-fluoroadenosine
  modified_base 10: mod_base = OTHER; note = 2'-fluoroguanosine
  modified_base 11: mod_base = OTHER; note = 2'-fluorouridine
  modified_base 12: mod_base = OTHER; note = 2'-O-methyladenosine
  modified_base 13: mod_base = cm
  modified_base 14: mod_base = gm
  modified_base 15: mod_base = OTHER; note = 2'-O-methyladenosine
  modified_base 16: mod_base = cm
  modified_base 17..18: mod_base = um
  modified_base 19: mod_base = cm
  modified_base 20: mod_base = gm
  modified_base 21: mod_base = um
  modified_base 1^2: mod_base = OTHER; note = phosphorothioate linkage
  modified_base 2^3: mod_base = OTHER; note = phosphorothioate linkage
  modified_base 19^20: mod_base = OTHER; note = phosphorothioate linkage
  modified_base 20^21: mod_base = OTHER; note = phosphorothioate linkage
cctctgcgagtacgacttcgt

SEQ ID NO: 12 - RNA, 23 nt, synthetic construct
  source 1..23: mol_type = other RNA
  modified_base 1: mod_base = OTHER; note = 2'-O-methyladenosine
  modified_base 2: mod_base = OTHER; note = 2'-fluorocytidine
  modified_base 3: mod_base = gm
  modified_base 4..5: mod_base = OTHER; note = 2'-O-methyladenosine
  modified_base 6: mod_base = gm
  modified_base 7: mod_base = um
  modified_base 8: mod_base = cm
  modified_base 9: mod_base = gm
  modified_base 10: mod_base = um
  modified_base 11: mod_base = OTHER; note = 2'-O-methyladenosine
  modified_base 12: mod_base = cm
  modified_base 13: mod_base = um
  modified_base 14: mod_base = OTHER; note = 2'-fluorocytidine
  modified_base 15: mod_base = gm
  modified_base 16: mod_base = OTHER; note = 2'-fluorocytidine
  modified_base 17: mod_base = OTHER; note = 2'-O-methyladenosine
  modified_base 18: mod_base = gm
  modified_base 20..21: mod_base = gm
  modified_base 19: mod_base = OTHER; note = 2'-O-methyladenosine
  modified_base 22: mod_base = um
  modified_base 23: mod_base = gm
  modified_base 1^2: mod_base = OTHER; note = phosphorothioate linkage
  modified_base 2^3: mod_base = OTHER; note = phosphorothioate linkage
  modified_base 21^22: mod_base = OTHER; note = phosphorothioate linkage
  modified_base 22^23: mod_base = OTHER; note = phosphorothioate linkage
acgaagtcgtactcgcagaggtg

SEQ ID NO: 13 - RNA, 21 nt, synthetic construct
  source 1..21: mol_type = other RNA
  modified_base 1: mod_base = um
  modified_base 2: mod_base = gm
  modified_base 3: mod_base = cm
  modified_base 4: mod_base = gm
  modified_base 5: mod_base = OTHER; note = 2'-O-methyladenosine
  modified_base 6: mod_base = gm
  modified_base 7: mod_base = OTHER; note = 2'-fluorouridine
  modified_base 8: mod_base = OTHER; note = 2'-O-methyladenosine
  modified_base 9: mod_base = OTHER; note = 2'-fluorocytidine
  modified_base 10: mod_base = OTHER; note = 2'-fluoroguanosine
  modified_base 11: mod_base = OTHER; note = 2'-fluoroadenosine
  modified_base 12: mod_base = cm
  modified_base 13..14: mod_base = um
  modified_base 15: mod_base = cm
  modified_base 16: mod_base = gm
  modified_base 17: mod_base = um
  modified_base 18: mod_base = cm
  modified_base 19..21: mod_base = OTHER; note = 2'-O-methyladenosine
  modified_base 1^2: mod_base = OTHER; note = phosphorothioate linkage
  modified_base 2^3: mod_base = OTHER; note = phosphorothioate linkage
  modified_base 19^20: mod_base = OTHER; note = phosphorothioate linkage
  modified_base 20^21: mod_base = OTHER; note = phosphorothioate linkage
tgcgagtacgacttcgtcaaa

SEQ ID NO: 14 - RNA, 23 nt, synthetic construct
  source 1..23: mol_type = other RNA
  modified_base 1: mod_base = um
  modified_base 2: mod_base = OTHER; note = 2'-fluorouridine
  modified_base 3: mod_base = um
  modified_base 4: mod_base = gm
  modified_base 5: mod_base = OTHER; note = 2'-O-methyladenosine
  modified_base 6: mod_base = cm
  modified_base 7: mod_base = gm
  modified_base 8..9: mod_base = OTHER; note = 2'-O-methyladenosine
  modified_base 10: mod_base = gm
  modified_base 11: mod_base = um
  modified_base 12: mod_base = cm
  modified_base 13: mod_base = gm
  modified_base 14: mod_base = OTHER; note = 2'-fluorouridine
  modified_base 15: mod_base = OTHER; note = 2'-O-methyladenosine
  modified_base 16: mod_base = OTHER; note = 2'-fluorocytidine
  modified_base 17: mod_base = um
  modified_base 18: mod_base = cm
  modified_base 19: mod_base = gm
  modified_base 20: mod_base = cm
  modified_base 21: mod_base = OTHER; note = 2'-O-methyladenosine
  modified_base 22: mod_base = gm
  modified_base 23: mod_base = OTHER; note = 2'-O-methyladenosine
  modified_base 1^2: mod_base = OTHER; note = phosphorothioate linkage
  modified_base 2^3: mod_base = OTHER; note = phosphorothioate linkage
  modified_base 21^22: mod_base = OTHER; note = phosphorothioate linkage
  modified_base 22^23: mod_base = OTHER; note = phosphorothioate linkage
tttgacgaagtcgtactcgcaga

SEQ ID NO: 15 - RNA, 21 nt, synthetic construct
  source 1..21: mol_type = other RNA
  modified_base 1: mod_base = gm
  modified_base 2..3: mod_base = cm
  modified_base 4: mod_base = um
  modified_base 5..6: mod_base = gm
  modified_base 7: mod_base = OTHER; note = 2'-fluoroadenosine
  modified_base 8: mod_base = cm
  modified_base 9: mod_base = OTHER; note = 2'-fluoroadenosine
  modified_base 10..11: mod_base = OTHER; note = 2'-fluorouridine
  modified_base 12: mod_base = OTHER; note = 2'-O-methyladenosine
  modified_base 13..14: mod_base = cm
  modified_base 15..16: mod_base = um
  modified_base 17..18: mod_base = cm
  modified_base 19: mod_base = gm
  modified_base 20: mod_base = cm
  modified_base 21: mod_base = um
  modified_base 1^2: mod_base = OTHER; note = phosphorothioate linkage
  modified_base 2^3: mod_base = OTHER; note = phosphorothioate linkage
  modified_base 19^20: mod_base = OTHER; note = phosphorothioate linkage
  modified_base 20^21: mod_base = OTHER; note = phosphorothioate linkage
gcctggacattaccttccgct

SEQ ID NO: 16 - RNA, 23 nt, synthetic construct
  source 1..23: mol_type = other RNA
  modified_base 1: mod_base = OTHER; note = 2'-O-methyladenosine
  modified_base 2: mod_base = OTHER; note = 2'-fluoroguanosine
  modified_base 3: mod_base = cm
  modified_base 4..5: mod_base = gm
  modified_base 6..7: mod_base = OTHER; note = 2'-O-methyladenosine
  modified_base 8..9: mod_base = gm
  modified_base 10: mod_base = um
  modified_base 11..12: mod_base = OTHER; note = 2'-O-methyladenosine
  modified_base 13: mod_base = um
  modified_base 14: mod_base = OTHER; note = 2'-fluoroguanosine
  modified_base 15: mod_base = um
  modified_base 16: mod_base = OTHER; note = 2'-fluorocytidine
  modified_base 17: mod_base = cm
  modified_base 18: mod_base = OTHER; note = 2'-O-methyladenosine
  modified_base 19..20: mod_base = gm
  modified_base 21: mod_base = cm
  modified_base 22: mod_base = um
  modified_base 23: mod_base = gm
  modified_base 1^2: mod_base = OTHER; note = phosphorothioate linkage
  modified_base 2^3: mod_base = OTHER; note = phosphorothioate linkage
  modified_base 21^22: mod_base = OTHER; note = phosphorothioate linkage
  modified_base 22^23: mod_base = OTHER; note = phosphorothioate linkage
agcggaaggtaatgtccaggctg

SEQ ID NO: 17 - RNA, 21 nt, synthetic construct
  source 1..21: mol_type = other RNA
  modified_base 1: mod_base = gm
  modified_base 2..3: mod_base = OTHER; note = 2'-O-methyladenosine
  modified_base 4: mod_base = gm
  modified_base 5..6: mod_base = cm
  modified_base 7: mod_base = OTHER; note = 2'-fluoroguanosine
  modified_base 8: mod_base = um
  modified_base 9: mod_base = OTHER; note = 2'-fluorouridine
  modified_base 10: mod_base = OTHER; note = 2'-fluorocytidine
  modified_base 11: mod_base = OTHER; note = 2'-fluoroadenosine
  modified_base 12: mod_base = cm
  modified_base 13..16: mod_base = gm
  modified_base 17..18: mod_base = um
  modified_base 19: mod_base = cm
  modified_base 20: mod_base = gm
  modified_base 21: mod_base = OTHER; note = 2'-O-methyladenosine
  modified_base 1^2: mod_base = OTHER; note = phosphorothioate linkage
  modified_base 2^3: mod_base = OTHER; note = phosphorothioate linkage
  modified_base 19^20: mod_base = OTHER; note = phosphorothioate linkage
  modified_base 20^21: mod_base = OTHER; note = phosphorothioate linkage
gaagccgttcacggggttcga

SEQ ID NO: 18 - RNA, 23 nt, synthetic construct
  source 1..23: mol_type = other RNA
  modified_base 1: mod_base = um
  modified_base 2: mod_base = OTHER; note = 2'-fluorocytidine
  modified_base 3: mod_base = gm
  modified_base 4..5: mod_base = OTHER; note = 2'-O-methyladenosine
  modified_base 6..9: mod_base = cm
  modified_base 10: mod_base = gm
  modified_base 11: mod_base = um
  modified_base 12: mod_base = gm
  modified_base 13: mod_base = OTHER; note = 2'-O-methyladenosine
  modified_base 14: mod_base = OTHER; note = 2'-fluoroadenosine
  modified_base 15: mod_base = cm
  modified_base 16: mod_base = OTHER; note = 2'-fluoroguanosine
  modified_base 17: mod_base = gm
  modified_base 18: mod_base = cm
  modified_base 19..20: mod_base = um
  modified_base 21: mod_base = cm
  modified_base 22: mod_base = um
  modified_base 23: mod_base = cm
  modified_base 1^2: mod_base = OTHER; note = phosphorothioate linkage
  modified_base 2^3: mod_base = OTHER; note = phosphorothioate linkage
  modified_base 21^22: mod_base = OTHER; note = phosphorothioate linkage
  modified_base 22^23: mod_base = OTHER; note = phosphorothioate linkage
tcgaaccccgtgaacggcttctc

SEQ ID NO: 19 - RNA, 21 nt, synthetic construct
  source 1..21: mol_type = other RNA
  modified_base 1: mod_base = um
  modified_base 2: mod_base = OTHER; note = 2'-O-methyladenosine
  modified_base 3: mod_base = cm
  modified_base 4: mod_base = gm
  modified_base 5: mod_base = um
  modified_base 6: mod_base = cm
  modified_base 7: mod_base = OTHER; note = 2'-fluorocytidine
  modified_base 8: mod_base = um
  modified_base 9: mod_base = OTHER; note = 2'-fluoroguanosine
  modified_base 10: mod_base = OTHER; note = 2'-fluorocytidine
  modified_base 11: mod_base = OTHER; note = 2'-fluoroadenosine
  modified_base 12..13: mod_base = cm
  modified_base 14: mod_base = gm
  modified_base 15: mod_base = um
  modified_base 16..17: mod_base = OTHER; note = 2'-O-methyladenosine
  modified_base 18: mod_base = cm
  modified_base 19..21: mod_base = OTHER; note = 2'-O-methyladenosine
  modified_base 1^2: mod_base = OTHER; note = phosphorothioate linkage
  modified_base 2^3: mod_base = OTHER; note = phosphorothioate linkage
  modified_base 19^20: mod_base = OTHER; note = phosphorothioate linkage
  modified_base 20^21: mod_base = OTHER; note = phosphorothioate linkage
tacgtcctgcaccgtaacaaa

SEQ ID NO: 20 - RNA, 23 nt, synthetic construct
  source 1..23: mol_type = other RNA
  modified_base 1: mod_base = um
  modified_base 2: mod_base = OTHER; note = 2'-fluorouridine
  modified_base 3: mod_base = um
  modified_base 4: mod_base = gm
  modified_base 5..6: mod_base = um
  modified_base 7: mod_base = OTHER; note = 2'-O-methyladenosine
  modified_base 8: mod_base = cm
  modified_base 9..10: mod_base = gm
  modified_base 11: mod_base = um
  modified_base 12: mod_base = gm
  modified_base 13: mod_base = cm
  modified_base 14: mod_base = OTHER; note = 2'-fluoroadenosine
  modified_base 15: mod_base = gm
  modified_base 16: mod_base = OTHER; note = 2'-fluoroguanosine
  modified_base 17: mod_base = OTHER; note = 2'-O-methyladenosine
  modified_base 18: mod_base = cm
  modified_base 19: mod_base = gm
  modified_base 20: mod_base = um
  modified_base 21: mod_base = OTHER; note = 2'-O-methyladenosine
  modified_base 22: mod_base = gm
  modified_base 23: mod_base = cm
  modified_base 1^2: mod_base = OTHER; note = phosphorothioate linkage
  modified_base 2^3: mod_base = OTHER; note = phosphorothioate linkage
  modified_base 21^22: mod_base = OTHER; note = phosphorothioate linkage
  modified_base 22^23: mod_base = OTHER; note = phosphorothioate linkage
tttgttacggtgcaggacgtagc

SEQ ID NO: 21 - RNA, 21 nt, synthetic construct
  source 1..21: mol_type = other RNA
  modified_base 1: mod_base = OTHER; note = 2'-O-methyladenosine
  modified_base 2: mod_base = gm
  modified_base 3: mod_base = cm
  modified_base 4..5: mod_base = um
  modified_base 6: mod_base = cm
  modified_base 7: mod_base = OTHER; note = 2'-fluorouridine
  modified_base 8: mod_base = cm
  modified_base 9: mod_base = OTHER; note = 2'-fluorocytidine
  modified_base 10: mod_base = OTHER; note = 2'-fluoroadenosine
  modified_base 11: mod_base = OTHER; note = 2'-fluorouridine
  modified_base 12: mod_base = cm
  modified_base 13..16: mod_base = um
  modified_base 17: mod_base = gm
  modified_base 18: mod_base = cm
  modified_base 19: mod_base = gm
  modified_base 20..21: mod_base = OTHER; note = 2'-O-methyladenosine
  modified_base 1^2: mod_base = OTHER; note = phosphorothioate linkage
  modified_base 2^3: mod_base = OTHER; note = phosphorothioate linkage
  modified_base 19^20: mod_base = OTHER; note = phosphorothioate linkage
  modified_base 20^21: mod_base = OTHER; note = phosphorothioate linkage
agcttctccatcttttgcgaa

SEQ ID NO: 22 - RNA, 23 nt, synthetic construct
  source 1..23: mol_type = other RNA
  modified_base 1: mod_base = um
  modified_base 2: mod_base = OTHER; note = 2'-fluorouridine
  modified_base 3: mod_base = cm
  modified_base 4: mod_base = gm
  modified_base 5: mod_base = cm
  modified_base 6..9: mod_base = OTHER; note = 2'-O-methyladenosine
  modified_base 10: mod_base = gm
  modified_base 11: mod_base = OTHER; note = 2'-O-methyladenosine
  modified_base 12: mod_base = um
  modified_base 13: mod_base = gm
  modified_base 14: mod_base = OTHER; note = 2'-fluoroguanosine
  modified_base 15: mod_base = OTHER; note = 2'-O-methyladenosine
  modified_base 16: mod_base = OTHER; note = 2'-fluoroguanosine
  modified_base 17..18: mod_base = OTHER; note = 2'-O-methyladenosine
  modified_base 19: mod_base = gm
  modified_base 20: mod_base = cm
  modified_base 21: mod_base = um
  modified_base 22: mod_base = gm
  modified_base 23: mod_base = um
  modified_base 1^2: mod_base = OTHER; note = phosphorothioate linkage
  modified_base 2^3: mod_base = OTHER; note = phosphorothioate linkage
  modified_base 21^22: mod_base = OTHER; note = phosphorothioate linkage
  modified_base 22^23: mod_base = OTHER; note = phosphorothioate linkage
ttcgcaaaagatggagaagctgt

SEQ ID NO: 23 - RNA, 21 nt, synthetic construct
  source 1..21: mol_type = other RNA
  modified_base 1: mod_base = um
  modified_base 2: mod_base = gm
  modified_base 3: mod_base = cm
  modified_base 4: mod_base = OTHER; note = 2'-O-methyladenosine
  modified_base 5..6: mod_base = cm
  modified_base 7: mod_base = OTHER; note = 2'-fluoroguanosine
  modified_base 8: mod_base = um
  modified_base 9..10: mod_base = OTHER; note = 2'-fluoroadenosine
  modified_base 11: mod_base = OTHER; note = 2'-fluorocytidine
  modified_base 12..13: mod_base = OTHER; note = 2'-O-methyladenosine
  modified_base 14: mod_base = gm
  modified_base 15: mod_base = cm
  modified_base 16: mod_base = gm
  modified_base 17: mod_base = cm
  modified_base 18: mod_base = OTHER; note = 2'-O-methyladenosine
  modified_base 19..20: mod_base = cm
  modified_base 21: mod_base = um
  modified_base 1^2: mod_base = OTHER; note = phosphorothioate linkage
  modified_base 2^3: mod_base = OTHER; note = phosphorothioate linkage
  modified_base 19^20: mod_base = OTHER; note = phosphorothioate linkage
  modified_base 20^21: mod_base = OTHER; note = phosphorothioate linkage
tgcaccgtaacaagcgcacct

SEQ ID NO: 24 - RNA, 23 nt, synthetic construct
  source 1..23: mol_type = other RNA
  modified_base 1: mod_base = OTHER; note = 2'-O-methyladenosine
  modified_base 2: mod_base = OTHER; note = 2'-fluoroguanosine
  modified_base 3: mod_base = gm
  modified_base 4: mod_base = um
  modified_base 5: mod_base = gm
  modified_base 6: mod_base = cm
  modified_base 7: mod_base = gm
  modified_base 8: mod_base = cm
  modified_base 9..10: mod_base = um
  modified_base 11: mod_base = gm
  modified_base 12..13: mod_base = um
  modified_base 14: mod_base = OTHER; note = 2'-fluoroadenosine
  modified_base 15: mod_base = cm
  modified_base 16: mod_base = OTHER; note = 2'-fluoroguanosine
  modified_base 17: mod_base = gm
  modified_base 18: mod_base = um
  modified_base 19: mod_base = gm
  modified_base 20: mod_base = cm
  modified_base 21: mod_base = OTHER; note = 2'-O-methyladenosine
  modified_base 22..23: mod_base = gm
  modified_base 1^2: mod_base = OTHER; note = phosphorothioate linkage
  modified_base 2^3: mod_base = OTHER; note = phosphorothioate linkage
  modified_base 21^22: mod_base = OTHER; note = phosphorothioate linkage
  modified_base 22^23: mod_base = OTHER; note = phosphorothioate linkage
aggtgcgcttgttacggtgcagg

SEQ ID NO: 25 - RNA, 21 nt, synthetic construct
  source 1..21: mol_type = other RNA
  modified_base 1: mod_base = gm
  modified_base 2: mod_base = cm
  modified_base 3: mod_base = um
  modified_base 4..5: mod_base = cm
  modified_base 6: mod_base = gm
  modified_base 7: mod_base = OTHER; note = 2'-fluoroadenosine
  modified_base 8: mod_base = cm
  modified_base 9: mod_base = OTHER; note = 2'-fluorouridine
  modified_base 10: mod_base = OTHER; note = 2'-fluoroadenosine
  modified_base 11: mod_base = OTHER; note = 2'-fluorocytidine
  modified_base 12: mod_base = um
  modified_base 13..14: mod_base = cm
  modified_base 15..16: mod_base = OTHER; note = 2'-O-methyladenosine
  modified_base 17: mod_base = cm
  modified_base 18: mod_base = gm
  modified_base 19: mod_base = OTHER; note = 2'-O-methyladenosine
  modified_base 20: mod_base = gm
  modified_base 21: mod_base = OTHER; note = 2'-O-methyladenosine
  modified_base 1^2: mod_base = OTHER; note = phosphorothioate linkage
  modified_base 2^3: mod_base = OTHER; note = phosphorothioate linkage
gctccgactactccaacgaga

SEQ ID NO: 26 - RNA, 21 nt, synthetic construct
  source 1..21: mol_type = other RNA
  modified_base 1: mod_base = um
  modified_base 2: mod_base = OTHER; note = 2'-O-methyladenosine
  modified_base 3: mod_base = um
  modified_base 4..5: mod_base = cm
  modified_base 6: mod_base = gm
  modified_base 7: mod_base = OTHER; note = 2'-fluoroadenosine
  modified_base 8: mod_base = um
  modified_base 9..10: mod_base = OTHER; note = 2'-fluoroguanosine
  modified_base 11: mod_base = OTHER; note = 2'-fluorocytidine
  modified_base 12: mod_base = gm
  modified_base 13..14: mod_base = cm
  modified_base 15: mod_base = OTHER; note = 2'-O-methyladenosine
  modified_base 16..17: mod_base = cm
  modified_base 18: mod_base = um
  modified_base 19..20: mod_base = OTHER; note = 2'-O-methyladenosine
  modified_base 21: mod_base = um
  modified_base 1^2: mod_base = OTHER; note = phosphorothioate linkage
  modified_base 2^3: mod_base = OTHER; note = phosphorothioate linkage
tatccgatggcgccacctaat

SEQ ID NO: 27 - RNA, 21 nt, synthetic construct
  source 1..21: mol_type = other RNA
  modified_base 1: mod_base = cm
  modified_base 2: mod_base = OTHER; note = 2'-O-methyladenosine
  modified_base 3..4: mod_base = cm
  modified_base 5: mod_base = gm
  modified_base 6: mod_base = um
  modified_base 7: mod_base = OTHER; note = 2'-fluoroadenosine
  modified_base 8: mod_base = OTHER; note = 2'-O-methyladenosine
  modified_base 9: mod_base = OTHER; note = 2'-fluorocytidine
  modified_base 10..11: mod_base = OTHER; note = 2'-fluoroadenosine
  modified_base 12: mod_base = gm
  modified_base 13: mod_base = cm
  modified_base 14: mod_base = gm
  modified_base 15: mod_base = cm
  modified_base 16: mod_base = OTHER; note = 2'-O-methyladenosine
  modified_base 17..18: mod_base = cm
  modified_base 19: mod_base = um
  modified_base 20: mod_base = gm
  modified_base 21: mod_base = OTHER; note = 2'-O-methyladenosine
  modified_base 1^2: mod_base = OTHER; note = phosphorothioate linkage
  modified_base 2^3: mod_base = OTHER; note = phosphorothioate linkage
caccgtaacaagcgcacctga

SEQ ID NO: 28 - RNA, 21 nt, synthetic construct
  source 1..21: mol_type = other RNA
  modified_base 1: mod_base = cm
  modified_base 2: mod_base = um
  modified_base 3: mod_base = OTHER; note = 2'-O-methyladenosine
  modified_base 4..5: mod_base = cm
  modified_base 6: mod_base = gm
  modified_base 7: mod_base = OTHER; note = 2'-fluorocytidine
  modified_base 8: mod_base = cm
  modified_base 9: mod_base = OTHER; note = 2'-fluorouridine
  modified_base 10: mod_base = OTHER; note = 2'-fluoroguanosine
  modified_base 11: mod_base = OTHER; note = 2'-fluorocytidine
  modified_base 12: mod_base = gm
  modified_base 13..14: mod_base = cm
  modified_base 15: mod_base = um
  modified_base 16: mod_base = cm
  modified_base 17: mod_base = um
  modified_base 18: mod_base = OTHER; note = 2'-O-methyladenosine
  modified_base 19: mod_base = cm
  modified_base 20..21: mod_base = um
  modified_base 1^2: mod_base = OTHER; note = phosphorothioate linkage
  modified_base 2^3: mod_base = OTHER; note = phosphorothioate linkage
ctaccgcctgcgcctctactt

SEQ ID NO: 29 - RNA, 21 nt, synthetic construct
  source 1..21: mol_type = other RNA
  modified_base 1..2: mod_base = cm
  modified_base 3: mod_base = gm
  modified_base 4: mod_base = um
  modified_base 5..6: mod_base = OTHER; note = 2'-O-methyladenosine
  modified_base 7: mod_base = OTHER; note = 2'-fluorocytidine
  modified_base 8: mod_base = OTHER; note = 2'-O-methyladenosine
  modified_base 9: mod_base = OTHER; note = 2'-fluoroadenosine
  modified_base 10: mod_base = OTHER; note = 2'-fluoroguanosine
  modified_base 11: mod_base = OTHER; note = 2'-fluorocytidine
  modified_base 12: mod_base = gm
  modified_base 13: mod_base = cm
  modified_base 14: mod_base = OTHER; note = 2'-O-methyladenosine
  modified_base 15..16: mod_base = cm
  modified_base 17: mod_base = um
  modified_base 18: mod_base = gm
  modified_base 19: mod_base = cm
  modified_base 20: mod_base = um
  modified_base 21: mod_base = OTHER; note = 2'-O-methyladenosine
  modified_base 1^2: mod_base = OTHER; note = phosphorothioate linkage
  modified_base 2^3: mod_base = OTHER; note = phosphorothioate linkage
ccgtaacaagcgcacctgcta

SEQ ID NO: 30 - RNA, 21 nt, synthetic construct
  source 1..21: mol_type = other RNA
  modified_base 1..2: mod_base = cm
  modified_base 3: mod_base = um
  modified_base 4: mod_base = cm
  modified_base 5: mod_base = um
  modified_base 6: mod_base = gm
  modified_base 7: mod_base = OTHER; note = 2'-fluorocytidine
  modified_base 8: mod_base = gm
  modified_base 9: mod_base = OTHER; note = 2'-fluoroadenosine
  modified_base 10: mod_base = OTHER; note = 2'-fluoroguanosine
  modified_base 11: mod_base = OTHER; note = 2'-fluorouridine
  modified_base 12: mod_base = OTHER; note = 2'-O-methyladenosine
  modified_base 13: mod_base = cm
  modified_base 14: mod_base = gm
  modified_base 15: mod_base = OTHER; note = 2'-O-methyladenosine
  modified_base 16: mod_base = cm
  modified_base 17..18: mod_base = um
  modified_base 19: mod_base = cm
  modified_base 20: mod_base = gm
  modified_base 21: mod_base = um
  modified_base 1^2: mod_base = OTHER; note = phosphorothioate linkage
  modified_base 2^3: mod_base = OTHER; note = phosphorothioate linkage
cctctgcgagtacgacttcgt

SEQ ID NO: 31 - RNA, 21 nt, synthetic construct
  source 1..21: mol_type = other RNA
  modified_base 1: mod_base = um
  modified_base 2: mod_base = gm
  modified_base 3: mod_base = cm
  modified_base 4: mod_base = gm
  modified_base 5: mod_base = OTHER; note = 2'-O-methyladenosine
  modified_base 6: mod_base = gm
  modified_base 7: mod_base = OTHER; note = 2'-fluorouridine
  modified_base 8: mod_base = OTHER; note = 2'-O-methyladenosine
  modified_base 9: mod_base = OTHER; note = 2'-fluorocytidine
  modified_base 10: mod_base = OTHER; note = 2'-fluoroguanosine
  modified_base 11: mod_base = OTHER; note = 2'-fluoroadenosine
  modified_base 12: mod_base = cm
  modified_base 13..14: mod_base = um
  modified_base 15: mod_base = cm
  modified_base 16: mod_base = gm
  modified_base 17: mod_base = um
  modified_base 18: mod_base = cm
  modified_base 19..21: mod_base = OTHER; note = 2'-O-methyladenosine
  modified_base 1^2: mod_base = OTHER; note = phosphorothioate linkage
  modified_base 2^3: mod_base = OTHER; note = phosphorothioate linkage
tgcgagtacgacttcgtcaaa

SEQ ID NO: 32 - RNA, 21 nt, synthetic construct
  source 1..21: mol_type = other RNA
  modified_base 1: mod_base = gm
  modified_base 2..3: mod_base = cm
  modified_base 4: mod_base = um
  modified_base 5..6: mod_base = gm
  modified_base 7: mod_base = OTHER; note = 2'-fluoroadenosine
  modified_base 8: mod_base = cm
  modified_base 9: mod_base = OTHER; note = 2'-fluoroadenosine
  modified_base 10..11: mod_base = OTHER; note = 2'-fluorouridine
  modified_base 12: mod_base = OTHER; note = 2'-O-methyladenosine
  modified_base 13..14: mod_base = cm
  modified_base 15..16: mod_base = um
  modified_base 17..18: mod_base = cm
  modified_base 19: mod_base = gm
  modified_base 20: mod_base = cm
  modified_base 21: mod_base = um
  modified_base 1^2: mod_base = OTHER; note = phosphorothioate linkage
  modified_base 2^3: mod_base = OTHER; note = phosphorothioate linkage
gcctggacattaccttccgct

SEQ ID NO: 33 - RNA, 21 nt, synthetic construct
  source 1..21: mol_type = other RNA
  modified_base 1: mod_base = gm
  modified_base 2..3: mod_base = OTHER; note = 2'-O-methyladenosine
  modified_base 4: mod_base = gm
  modified_base 5..6: mod_base = cm
  modified_base 7: mod_base = OTHER; note = 2'-fluoroguanosine
  modified_base 8: mod_base = um
  modified_base 9: mod_base = OTHER; note = 2'-fluorouridine
  modified_base 10: mod_base = OTHER; note = 2'-fluorocytidine
  modified_base 11: mod_base = OTHER; note = 2'-fluoroadenosine
  modified_base 12: mod_base = cm
  modified_base 13..16: mod_base = gm
  modified_base 17..18: mod_base = um
  modified_base 19: mod_base = cm
  modified_base 20: mod_base = gm
  modified_base 21: mod_base = OTHER; note = 2'-O-methyladenosine
  modified_base 1^2: mod_base = OTHER; note = phosphorothioate linkage
  modified_base 2^3: mod_base = OTHER; note = phosphorothioate linkage
gaagccgttcacggggttcga

SEQ ID NO: 34 - RNA, 21 nt, synthetic construct
  source 1..21: mol_type = other RNA
  modified_base 1: mod_base = um
  modified_base 2: mod_base = OTHER; note = 2'-O-methyladenosine
  modified_base 3: mod_base = cm
  modified_base 4: mod_base = gm
  modified_base 5: mod_base = um
  modified_base 6: mod_base = cm
  modified_base 7: mod_base = OTHER; note = 2'-fluorocytidine
  modified_base 8: mod_base = um
  modified_base 9: mod_base = OTHER; note = 2'-fluoroguanosine
  modified_base 10: mod_base = OTHER; note = 2'-fluorocytidine
  modified_base 11: mod_base = OTHER; note = 2'-fluoroadenosine
  modified_base 12..13: mod_base = cm
  modified_base 14: mod_base = gm
  modified_base 15: mod_base = um
  modified_base 16..17: mod_base = OTHER; note = 2'-O-methyladenosine
  modified_base 18: mod_base = cm
  modified_base 19..21: mod_base = OTHER; note = 2'-O-methyladenosine
  modified_base 1^2: mod_base = OTHER; note = phosphorothioate linkage
  modified_base 2^3: mod_base = OTHER; note = phosphorothioate linkage
tacgtcctgcaccgtaacaaa

SEQ ID NO: 35 - RNA, 21 nt, synthetic construct
  source 1..21: mol_type = other RNA
  modified_base 1: mod_base = OTHER; note = 2'-O-methyladenosine
  modified_base 2: mod_base = gm
  modified_base 3: mod_base = cm
  modified_base 4..5: mod_base = um
  modified_base 6: mod_base = cm
  modified_base 7: mod_base = OTHER; note = 2'-fluorouridine
  modified_base 8: mod_base = cm
  modified_base 9: mod_base = OTHER; note = 2'-fluorocytidine
  modified_base 10: mod_base = OTHER; note = 2'-fluoroadenosine
  modified_base 11: mod_base = OTHER; note = 2'-fluorouridine
  modified_base 12: mod_base = cm
  modified_base 13..16: mod_base = um
  modified_base 17: mod_base = gm
  modified_base 18: mod_base = cm
  modified_base 19: mod_base = gm
  modified_base 20..21: mod_base = OTHER; note = 2'-O-methyladenosine
  modified_base 1^2: mod_base = OTHER; note = phosphorothioate linkage
  modified_base 2^3: mod_base = OTHER; note = phosphorothioate linkage
agcttctccatcttttgcgaa

SEQ ID NO: 36 - RNA, 21 nt, synthetic construct
  source 1..21: mol_type = other RNA
  modified_base 1: mod_base = um
  modified_base 2: mod_base = gm
  modified_base 3: mod_base = cm
  modified_base 4: mod_base = OTHER; note = 2'-O-methyladenosine
  modified_base 5..6: mod_base = cm
  modified_base 7: mod_base = OTHER; note = 2'-fluoroguanosine
  modified_base 8: mod_base = um
  modified_base 9..10: mod_base = OTHER; note = 2'-fluoroadenosine
  modified_base 11: mod_base = OTHER; note = 2'-fluorocytidine
  modified_base 12..13: mod_base = OTHER; note = 2'-O-methyladenosine
  modified_base 14: mod_base = gm
  modified_base 15: mod_base = cm
  modified_base 16: mod_base = gm
  modified_base 17: mod_base = cm
  modified_base 18: mod_base = OTHER; note = 2'-O-methyladenosine
  modified_base 19..20: mod_base = cm
  modified_base 21: mod_base = um
  modified_base 1^2: mod_base = OTHER; note = phosphorothioate linkage
  modified_base 2^3: mod_base = OTHER; note = phosphorothioate linkage
tgcaccgtaacaagcgcacct

SEQ ID NO: 37 - RNA, 21 nt, synthetic construct
  source 1..21: mol_type = other RNA
gctccgactactccaacgaga

SEQ ID NO: 38 - RNA, 23 nt, synthetic construct
  source 1..23: mol_type = other RNA
tctcgttggagtagtcggagcgg

SEQ ID NO: 39 - RNA, 21 nt, synthetic construct
  source 1..21: mol_type = other RNA
tatccgatggcgccacctaat

SEQ ID NO: 40 - RNA, 23 nt, synthetic construct
  source 1..23: mol_type = other RNA
attaggtggcgccatcggataag

SEQ ID NO: 41 - RNA, 21 nt, synthetic construct
  source 1..21: mol_type = other RNA
caccgtaacaagcgcacctga

SEQ ID NO: 42 - RNA, 23 nt, synthetic construct
  source 1..23: mol_type = other RNA
tcaggtgcgcttgttacggtgca

SEQ ID NO: 43 - RNA, 21 nt, synthetic construct
  source 1..21: mol_type = other RNA
ctaccgcctgcgcctctactt

SEQ ID NO: 44 - RNA, 23 nt, synthetic construct
  source 1..23: mol_type = other RNA
aagtagaggcgcaggcggtagcc

SEQ ID NO: 45 - RNA, 21 nt, synthetic construct
  source 1..21: mol_type = other RNA
ccgtaacaagcgcacctgcta

SEQ ID NO: 46 - RNA, 23 nt, synthetic construct
  source 1..23: mol_type = other RNA
tagcaggtgcgcttgttacggtg

SEQ ID NO: 47 - RNA, 21 nt, synthetic construct
  source 1..21: mol_type = other RNA
cctctgcgagtacgacttcgt

SEQ ID NO: 48 - RNA, 23 nt, synthetic construct
  source 1..23: mol_type = other RNA
acgaagtcgtactcgcagaggtg

SEQ ID NO: 49 - RNA, 21 nt, synthetic construct
  source 1..21: mol_type = other RNA
tgcgagtacgacttcgtcaaa

SEQ ID NO: 50 - RNA, 23 nt, synthetic construct
  source 1..23: mol_type = other RNA
tttgacgaagtcgtactcgcaga

SEQ ID NO: 51 - RNA, 21 nt, synthetic construct
  source 1..21: mol_type = other RNA
gcctggacattaccttccgct

SEQ ID NO: 52 - RNA, 23 nt, synthetic construct
  source 1..23: mol_type = other RNA
agcggaaggtaatgtccaggctg

SEQ ID NO: 53 - RNA, 21 nt, synthetic construct
  source 1..21: mol_type = other RNA
gaagccgttcacggggttcga

SEQ ID NO: 54 - RNA, 23 nt, synthetic construct
  source 1..23: mol_type = other RNA
tcgaaccccgtgaacggcttctc

SEQ ID NO: 55 - RNA, 21 nt, synthetic construct
  source 1..21: mol_type = other RNA
tacgtcctgcaccgtaacaaa

SEQ ID NO: 56 - RNA, 23 nt, synthetic construct
  source 1..23: mol_type = other RNA
tttgttacggtgcaggacgtagc

SEQ ID NO: 57 - RNA, 21 nt, synthetic construct
  source 1..21: mol_type = other RNA
ctgcaccgtaacaagcgcacc

SEQ ID NO: 58 - RNA, 23 nt, synthetic construct
  source 1..23: mol_type = other RNA
ggtgcgcttgttacggtgcagga

SEQ ID NO: 59 - RNA, 21 nt, synthetic construct
  source 1..21: mol_type = other RNA
tctgcgagtacgacttcgtca

SEQ ID NO: 60 - RNA, 23 nt, synthetic construct
  source 1..23: mol_type = other RNA
tgacgaagtcgtactcgcagagg

SEQ ID NO: 61 - RNA, 21 nt, synthetic construct
  source 1..21: mol_type = other RNA
agcctggacattaccttccgc

SEQ ID NO: 62 - RNA, 23 nt, synthetic construct
  source 1..23: mol_type = other RNA
gcggaaggtaatgtccaggctgg

SEQ ID NO: 63 - RNA, 21 nt, synthetic construct
  source 1..21: mol_type = other RNA
gctacgtcctgcaccgtaaca

SEQ ID NO: 64 - RNA, 23 nt, synthetic construct
  source 1..23: mol_type = other RNA
tgttacggtgcaggacgtagcct

SEQ ID NO: 65 - RNA, 21 nt, synthetic construct
  source 1..21: mol_type = other RNA
tggacattaccttccgctccg

SEQ ID NO: 66 - RNA, 23 nt, synthetic construct
  source 1..23: mol_type = other RNA
cggagcggaaggtaatgtccagg

SEQ ID NO: 67 - RNA, 21 nt, synthetic construct
  source 1..21: mol_type = other RNA
ctccgactactccaacgagaa

SEQ ID NO: 68 - RNA, 23 nt, synthetic construct
  source 1..23: mol_type = other RNA
ttctcgttggagtagtcggagcg

SEQ ID NO: 69 - RNA, 21 nt, synthetic construct
  source 1..21: mol_type = other RNA
agaagccgttcacggggttcg

SEQ ID NO: 70 - RNA, 23 nt, synthetic construct
  source 1..23: mol_type = other RNA
cgaaccccgtgaacggcttctcg

SEQ ID NO: 71 - RNA, 21 nt, synthetic construct
  source 1..21: mol_type = other RNA
agcttctccatcttttgcgaa

SEQ ID NO: 72 - RNA, 23 nt, synthetic construct
  source 1..23: mol_type = other RNA
ttcgcaaaagatggagaagctgt

SEQ ID NO: 73 - RNA, 21 nt, synthetic construct
  source 1..21: mol_type = other RNA
cctggacattaccttccgctc

SEQ ID NO: 74 - RNA, 23 nt, synthetic construct
  source 1..23: mol_type = other RNA
gagcggaaggtaatgtccaggct

SEQ ID NO: 75 - RNA, 21 nt, synthetic construct
  source 1..21: mol_type = other RNA
tccgactactccaacgagaag

SEQ ID NO: 76 - RNA, 23 nt, synthetic construct
  source 1..23: mol_type = other RNA
cttctcgttggagtagtcggagc

SEQ ID NO: 77 - RNA, 21 nt, synthetic construct
  source 1..21: mol_type = other RNA
tgcaccgtaacaagcgcacct

SEQ ID NO: 78 - RNA, 23 nt, synthetic construct
  source 1..23: mol_type = other RNA
aggtgcgcttgttacggtgcagg

SEQ ID NO: 79 - RNA, 21 nt, synthetic construct
  source 1..21: mol_type = other RNA
cgtcctgcaccgtaacaagcg

SEQ ID NO: 80 - RNA, 23 nt, synthetic construct
  source 1..23: mol_type = other RNA
cgcttgttacggtgcaggacgta

SEQ ID NO: 81 - RNA, 21 nt, synthetic construct
  source 1..21: mol_type = other RNA
atccgatggcgccacctaatg

SEQ ID NO: 82 - RNA, 23 nt, synthetic construct
  source 1..23: mol_type = other RNA
cattaggtggcgccatcggataa

SEQ ID NO: 83 - RNA, 21 nt, synthetic construct
  source 1..21: mol_type = other RNA
ctgcaccccccggctaccgcc

SEQ ID NO: 84 - RNA, 23 nt, synthetic construct
  source 1..23: mol_type = other RNA
ggcggtagccggggggtgcagtc

SEQ ID NO: 85 - RNA, 21 nt, synthetic construct
  source 1..21: mol_type = other RNA
taactatattccctggatcga

SEQ ID NO: 86 - RNA, 23 nt, synthetic construct
  source 1..23: mol_type = other RNA
tcgatccagggaatatagttaat

SEQ ID NO: 87 - RNA, 21 nt, synthetic construct
  source 1..21: mol_type = other RNA
aggctacgtcctgcaccgtaa

SEQ ID NO: 88 - RNA, 23 nt, synthetic construct
  source 1..23: mol_type = other RNA
ttacggtgcaggacgtagcctgc

SEQ ID NO: 89 - RNA, 21 nt, synthetic construct
  source 1..21: mol_type = other RNA
ggctacgtcctgcaccgtaac

SEQ ID NO: 90 - RNA, 23 nt, synthetic construct
  source 1..23: mol_type = other RNA
gttacggtgcaggacgtagcctg

SEQ ID NO: 91 - RNA, 21 nt, synthetic construct
  source 1..21: mol_type = other RNA
aagccgttcacggggttcgag

SEQ ID NO: 92 - RNA, 23 nt, synthetic construct
  source 1..23: mol_type = other RNA
ctcgaaccccgtgaacggcttct

SEQ ID NO: 93 - RNA, 21 nt, synthetic construct
  source 1..21: mol_type = other RNA
tgtgtggctcggtggccaccc

SEQ ID NO: 94 - RNA, 23 nt, synthetic construct
  source 1..23: mol_type = other RNA
gggtggccaccgagccacacaga

SEQ ID NO: 95 - RNA, 21 nt, synthetic construct
  source 1..21: mol_type = other RNA
cttatccgatggcgccaccta

SEQ ID NO: 96 - RNA, 23 nt, synthetic construct
  source 1..23: mol_type = other RNA
taggtggcgccatcggataaggg

SEQ ID NO: 97 - RNA, 21 nt, synthetic construct
  source 1..21: mol_type = other RNA
tccgatggcgccacctaatgg

SEQ ID NO: 98 - RNA, 23 nt, synthetic construct
  source 1..23: mol_type = other RNA
ccattaggtggcgccatcggata

SEQ ID NO: 99 - RNA, 21 nt, synthetic construct
  source 1..21: mol_type = other RNA
ccgatggcgccacctaatggc

SEQ ID NO: 100 - RNA, 23 nt, synthetic construct
  source 1..23: mol_type = other RNA
gccattaggtggcgccatcggat

SEQ ID NO: 101 - RNA, 21 nt, synthetic construct
  source 1..21: mol_type = other RNA
gagtggagtacatcacaggtc

SEQ ID NO: 102 - RNA, 23 nt, synthetic construct
  source 1..23: mol_type = other RNA
gacctgtgatgtactccactcgg

SEQ ID NO: 103 - DNA, 20 bp, synthetic construct
  source 1..20: mol_type = other DNA
gatttggtcgtattgggcgc

SEQ ID NO: 104 - DNA, 20 bp, synthetic construct
  source 1..20: mol_type = other DNA
ttcccgttctcagccttgac

SEQ ID NO: 105 - DNA, 20 bp, synthetic construct
  source 1..20: mol_type = other DNA
cccagtctgtgagcctgttt

SEQ ID NO: 106 - DNA, 20 bp, synthetic construct
  source 1..20: mol_type = other DNA
gcagctgttaggacccagtt